European Patent Application EP 4 582 534 A1, published July 9, 2025. Title: ナイーブ型多能性幹細胞の製造方法. Applicant: 国立大学法人京都大学. Application JP. The sequence listing filed with the application follows.

SEQUENCE LISTING (15 sequences)

SEQ ID NO: 1 - RNA, 22 nt, Homo sapiens
  source 1..22: mol_type = other RNA
tgaggtagtaagttgtattgtt

SEQ ID NO: 2 - RNA, 22 nt, Homo sapiens
  source 1..22: mol_type = other RNA
tgaggtagtaggttgtatagtt

SEQ ID NO: 3 - RNA, 22 nt, Homo sapiens
  source 1..22: mol_type = other RNA
tgaggtagtaggttgtgtggtt

SEQ ID NO: 4 - RNA, 22 nt, Homo sapiens
  source 1..22: mol_type = other RNA
tgaggtagtaggttgtatggtt

SEQ ID NO: 5 - RNA, 22 nt, Homo sapiens
  source 1..22: mol_type = other RNA
tgaggtaggaggttgtatagtt

SEQ ID NO: 6 - RNA, 22 nt, Homo sapiens
  source 1..22: mol_type = other RNA
tgaggtagtagattgtatagtt

SEQ ID NO: 7 - RNA, 22 nt, Homo sapiens
  source 1..22: mol_type = other RNA
tgaggtagtagtttgtacagtt

SEQ ID NO: 8 - RNA, 22 nt, Homo sapiens
  source 1..22: mol_type = other RNA
tgaggtagtagtttgtgctgtt

SEQ ID NO: 9 - DNA, 37 bp, synthetic construct
  misc_feature 1..37: note = KEC001_Rev5UTR
  source 1..37: mol_type = other DNA
catggtggcgaccggtgtcttatatttcttcttactc

SEQ ID NO: 10 - DNA, 87 bp, synthetic construct
  misc_feature 1..87: note = KEC062_IVT_5prime_UTR
  source 1..87: mol_type = other DNA
cagtgaattgtaatacgactcactatagggcgaattaagagagaaaagaagagtaagaagaaatataagacaccggtcgccaccatg

SEQ ID NO: 11 - DNA, 28 bp, synthetic construct
  misc_feature 1..28: note = KEC876_TAP_T7_1G
  source 1..28: mol_type = other DNA
cagtgaattgtaatacgactcactatag

SEQ ID NO: 12 - DNA, 92 bp, synthetic construct
  misc_feature 1..92: note = KEC063_IVT_3prime_UTR
  source 1..92: mol_type = other DNA
tctagaccttctgcggggcttgccttctggccatgcccttcttctctcccttgcacctgtacctcttggtctttgaataaagcctgagtagg

SEQ ID NO: 13 - DNA, 48 bp, synthetic construct
  misc_feature 1..48: note = KEC065_Rev3UTR2T20
  source 1..48: mol_type = other DNA
ttttttttttttttttttttcctactcaggctttattcaaagaccaag

SEQ ID NO: 14 - DNA, 139 bp, synthetic construct
  misc_feature 1..139: note = KEC883_3UTR120A
  source 1..139: mol_type = other DNA
ttttttttttttttttttttttttttttttttttttttttttttttttttttttttttttttttttttttttttttttttttttttttttttttttttttttttttttttttttttttttcctactcaggctttattca

SEQ ID NO: 15 - DNA, 51 bp, synthetic construct
  misc_feature 1..51: note = YF0771-T7_5UTR_fwd
  source 1..51: mol_type = other DNA
attgtaatacgactcactatagggcgaattaagagagaaaagaagagtaag